European Patent Application EP 4 368 640 A1, published May 15, 2024. Title: CD19 ANTIBODY AND APPLICATION THEREOF. Applicant: 先声再明医药有限公司. Application EP. The sequence listing filed with the application follows.

SEQUENCE LISTING (449 sequences)

SEQ ID NO: 1 - protein, 450 aa, synthetic construct
EVKLQESGPGLVAPSQSLSVTCTVSGVSLPDYGVSWIRQPPRKGLEWLGVIWGSETTYYNSALKSRLTIIKDNSKSQVFLKMNSLQTDDTAIYYCAKHYYYGGSYAMDYWGQGTSVTVSSASTKGPSVFPLAPSSKSTSGGTAALGCLVKDYFPEPVTVSWNSGALTSGVHTFPAVLQSSGLYSLSSVVTVPSSSLGTQTYICNVNHKPSNTKVDKKVEPKSCDKTHTCPPCPAPELLGGPSVFLFPPKPKDTLMISRTPEVTCVVVDVSHEDPEVKFNWYVDGVEVHNAKTKPREEQYNSTYRVVSVLTVLHQDWLNGKEYKCKVSNKALPAPIEKTISKAKGQPREPQVYTLPPSREEMTKNQVSLTCLVKGFYPSDIAVEWESNGQPENNYKTTPPVLDSDGSFFLYSKLTVDKSRWQQGNVFSCSVMHEALHNHYTQKSLSLSPGK

SEQ ID NO: 2 - protein, 444 aa, synthetic construct
EVKLQESGPGLVAPSQSLSVTCTVSGVSLPDYGVSWIRQPPRKGLEWLGVIWGSETTYYNSALKSRLTIIKDNSKSQVFLKMNSLQTDDTAIYYCAKHYYYGGSYAMDYWGQGTSVTVSSAKTTPPSVYPLAPGSAAQTNSMVTLGCLVKGYFPEPVTVTWNSGSLSSGVHTFPAVLQSDLYTLSSSVTVPSSTWPSETVTCNVAHPASSTKVDKKIVPRDCGCKPCICTVPEVSSVFIFPPKPKDVLTITLTPKVTCVVVDISKDDPEVQFSWFVDDVEVHTAQTQPREEQFNSTFRSVSELPIMHQDWLNGKEFKCRVNSAAFPAPIEKTISKTKGRPKAPQVYTIPPPKEQMAKDKVSLTCMITDFFPEDITVEWQWNGQPAENYKNTQPIMDTDGSYFVYSKLNVQKSNWEAGNTFTCSVLHEGLHNHHTEKSLSHSPGK

SEQ ID NO: 3 - protein, 214 aa, synthetic construct
DIQMTQTTSSLSASLGDRVTISCRASQDISKYLNWYQQKPDGTVKLLIYHTSRLHSGVPSRFSGSGSGTDYSLTISNLEQEDIATYFCQQGNTLPYTFGGGTKLEITRTVAAPSVFIFPPSDEQLKSGTASVVCLLNNFYPREAKVQWKVDNALQSGNSQESVTEQDSKDSTYSLSSTLTLSKADYEKHKVYACEVTHQGLSSPVTKSFNRGEC

SEQ ID NO: 4 - protein, 214 aa, synthetic construct
DIQMTQTTSSLSASLGDRVTISCRASQDISKYLNWYQQKPDGTVKLLIYHTSRLHSGVPSRFSGSGSGTDYSLTISNLEQEDIATYFCQQGNTLPYTFGGGTKLEITRADAAPTVSIFPPSSEQLTSGGASVVCFLNNFYPKDINVKWKIDGSERQNGVLNSWTDQDSKDSTYSMSSTLTLTKDEYERHNSYTCEATHKTSTSPIVKSFNRNEC

SEQ ID NO: 5 - protein, 452 aa, synthetic construct
EVQLVQSGAEVKKPGESLKISCKGSGYSFTSYWIGWVRQMPGKGLEWMGIIYPGDSDTRYSPSFQGQVTISADKSISTAYLQWSSLKASDTAMYYCARGVSGIYNLHGFDIWGQGTLVTVSSASTKGPSVFPLAPSSKSTSGGTAALGCLVKDYFPEPVTVSWNSGALTSGVHTFPAVLQSSGLYSLSSVVTVPSSSLGTQTYICNVNHKPSNTKVDKKVEPKSCDKTHTCPPCPAPELLGGPSVFLFPPKPKDTLMISRTPEVTCVVVDVSHEDPEVKFNWYVDGVEVHNAKTKPREEQYNSTYRVVSVLTVLHQDWLNGKEYKCKVSNKALPAPIEKTISKAKGQPREPQVYTLPPSREEMTKNQVSLTCLVKGFYPSDIAVEWESNGQPENNYKTTPPVLDSDGSFFLYSKLTVDKSRWQQGNVFSCSVMHEALHNHYTQKSLSLSPGK

SEQ ID NO: 6 - protein, 446 aa, synthetic construct
EVQLVQSGAEVKKPGESLKISCKGSGYSFTSYWIGWVRQMPGKGLEWMGIIYPGDSDTRYSPSFQGQVTISADKSISTAYLQWSSLKASDTAMYYCARGVSGIYNLHGFDIWGQGTLVTVSSAKTTPPSVYPLAPGSAAQTNSMVTLGCLVKGYFPEPVTVTWNSGSLSSGVHTFPAVLQSDLYTLSSSVTVPSSTWPSETVTCNVAHPASSTKVDKKIVPRDCGCKPCICTVPEVSSVFIFPPKPKDVLTITLTPKVTCVVVDISKDDPEVQFSWFVDDVEVHTAQTQPREEQFNSTFRSVSELPIMHQDWLNGKEFKCRVNSAAFPAPIEKTISKTKGRPKAPQVYTIPPPKEQMAKDKVSLTCMITDFFPEDITVEWQWNGQPAENYKNTQPIMDTDGSYFVYSKLNVQKSNWEAGNTFTCSVLHEGLHNHHTEKSLSHSPGK

SEQ ID NO: 7 - protein, 215 aa, synthetic construct
DIQMTQSPSSLSASVGDRVTITCRASQSISSYLNWYQQKPGKAPKLLIYAASSLQSGVPSRFSGSGSGTDFTLTISSLQPEDFATYYCQQGRFGSPFTFGQGTKVEIKRTVAAPSVFIFPPSDEQLKSGTASVVCLLNNFYPREAKVQWKVDNALQSGNSQESVTEQDSKDSTYSLSSTLTLSKADYEKHKVYACEVTHQGLSSPVTKSFNRGEC

SEQ ID NO: 8 - protein, 215 aa, synthetic construct
DIQMTQSPSSLSASVGDRVTITCRASQSISSYLNWYQQKPGKAPKLLIYAASSLQSGVPSRFSGSGSGTDFTLTISSLQPEDFATYYCQQGRFGSPFTFGQGTKVEIKRADAAPTVSIFPPSSEQLTSGGASVVCFLNNFYPKDINVKWKIDGSERQNGVLNSWTDQDSKDSTYSMSSTLTLTKDEYERHNSYTCEATHKTSTSPIVKSFNRNEC

SEQ ID NO: 9 - protein, 120 aa, synthetic construct
EVQLQQSGPELVKPGASVKMSCKASGYTFTDYVMHWVRQTPGQGLEWIGYFNPYNDGTNYNEKFKVKATLTSDKSSTTAYMELSSLTSEDSAVYYCARGVYYYGRDFDYWGQGTTLTVSS

SEQ ID NO: 10 - protein, 112 aa, synthetic construct
DVVLTQTPLSLPVSLGDQASISCRSSQSLENSNGNSYLNWYLQKPGQSPQLLIYRVSNRFSGVLDRFSGSGSGTDFTLKISRVEAEDLGVYFCLQITHVPWTFGGGTKLEIK

SEQ ID NO: 11 - protein, 120 aa, synthetic construct
QVQLKESGPGLVAPSQSLSITCTVSGFSLTDYGVSWIRQSPGKGLEWLGVIWGSGDTYYNSVLESRLSINKDNSKNQVFLKMNSLQTDDAAMYFCAKHSYYGGSFAMDYWGQGTSVTVSS

SEQ ID NO: 12 - protein, 107 aa, synthetic construct
DIQMTQTTSSLSASLGDRVTISCRASQDISNYLNWYQQKPDGTVKLLIYYTSRLHSGVPSRFSGSGSGTDYSLTISNLEQEDIATYFCQQGKTLPWTFGGGTKLEIK

SEQ ID NO: 13 - protein, 119 aa, synthetic construct
DVQLQESGPGLAKLSQSLSLTCSVTGYSITSGYYWNWIRQFPGNKLEWMGHISYDGNNNYNPSLKNRISITRDTSKNQFFLKLNSVTTEDTATYYCARENYSNYYFDYWGQGTTLTVSS

SEQ ID NO: 14 - protein, 111 aa, synthetic construct
DIVLTQSPASLAVSLGQRATISCRASQSVSKSSYTYIHWYQQKPGQPPKLLIKYASILQSGVPARFSGSGSGTDFTLNFHPVEEEDTATYYCQHSWEIPYTFGGGTKLEIK

SEQ ID NO: 15 - protein, 118 aa, synthetic construct
QAQLQQSGPELVKPGASVKISCKASGYAFSGSWMNWVQQRPGKGLEWIGRIYPGDGDTYYNGKFKDKAILTADKSSSTAYMQLSSLTSEDSAVYFCAQLRYRYVMDYWGQGTSVTVSS

SEQ ID NO: 16 - protein, 111 aa, synthetic construct
DIVLTQSPASLAVSLGQRATISCRASESVSIHGSHLMHWYQQKPGQPPRLLIYAASNLESGVPARFSGSGSETDFTLNIHPVEEEDAATYFCQQGIKDPYTFGGGTKLEIK

SEQ ID NO: 17 - protein, 120 aa, synthetic construct
DVQLQESGPGLMKPSQSLSLTCSVTGYSITSGYYWNWIRQFPGNKLEWMGYISYDGSNNYNPSLKNRFSITRDTSKNQFFLKLNSVTTEDTATYYCARRKLTGGPYFDYWGQGTTLTVSS

SEQ ID NO: 18 - protein, 111 aa, unidentified
DIVLTQSPASLAVTLGQRATISCRASESVSFHGFHIMHWYQQKPGQPPKLLIYAASHLVSGVPDRFSGSGSETDFTLNIHPVEEEDAAAYFCQQSVEDPWTFGGGTKLEIK

SEQ ID NO: 19 - protein, 120 aa, synthetic construct
EFQLQQSGPELVKPGASVKISCKASDYSFTDYNMNWVKQSNGASLEWIGIINPNFGSTSYNQKFKGKATLTVDQSSSTAFMQLNSLTSEDSAVYYCARSEYYGSSGFAYWGQGTLVTVSA

SEQ ID NO: 20 - protein, 112 aa, synthetic construct
DVVVTQTPLSLPVSFGDQVSISCRSSQSLVNSYGNTYLSWYLHKPGQSPQLLIYGISNRFSGVPDRFSGSGSGTDFTLKITTIKPEDLGMYYCLQGTHQPWTFGGGTKLEIK

SEQ ID NO: 21 - protein, 118 aa, unidentified
QAQLQQSGPELVKPGASVKISCKASGYAFSGSWMNWVQQRPGKGLEWIGRIYPGDGDTYYSGKFKDKAILTADTSSSTAYMQLSSLTSEDSAVYFCAQLRSRYVMDYWGQGASVTVSS

SEQ ID NO: 22 - protein, 111 aa, synthetic construct
DIVLTQSPASLAVSLGQRATISCRASESVSIHGTHLMHWYQQKPGQPPRLLIYAASNLESGVPARFSGSGSETDFTLNIHPVEEEDAATYFCQQGIDDPYTFGGGTKLEIK

SEQ ID NO: 23 - protein, 121 aa, synthetic construct
EVQLQQSGPELVKPGASVKISCKASGYTFTDYHINWVKQSHGKSPEWIGDINPNNGGTTYNQKFKDKATLTVDKSSSTAFMELRSLTSEDSAVYYCARFITTVVAWYFDVWGTGTTVTVSS

SEQ ID NO: 24 - protein, 107 aa, synthetic construct
DIQMTQSPASLSVSVGETVTITCRASENIYSNLAWYQQKQGKSPQLLVYAATNLADGVPSRFSGSGSGTQYSLKINSLQSEDFGNYYCQRFWDTPRTFGGGTKLEIK

SEQ ID NO: 25 - protein, 114 aa, synthetic construct
QVQLQQSGAELVRPGASVTLSCKASGYTFTDYEMHWVKQTPVHGLEWIGGIAPETGLTTYNQKFEDKAILTADKSSRTAYMELRSLTSEDSAVYFCNPNNYGLWGTGTTVTVSS

SEQ ID NO: 26 - protein, 112 aa, synthetic construct
DVVMTQTPLTLSVTIGQPASISCKSSQSLLDSNGKTYLNWLLQRPGQSPKRLIYLVSKLDSGVPDRVTGSGSGTDFTLKISRVEAEDLGVYYCWQGTHFPWTFGGGTKLEIK

SEQ ID NO: 27 - protein, 113 aa, synthetic construct
EFQLQQSGPELVKPGASVKISCKASGYSFTDYNMNWVKQSNGKSLEWIGTINPNYITSYNQKFKGKATLTVDQSSSTAYMQLNSLTSEDSAVYYCAGDYKGYWGQGTTLTVSS

SEQ ID NO: 28 - protein, 112 aa, synthetic construct
DVVMTQTPLTLSVTIGQPASISCKSSQNLLDSDGKTYLNWLLQRPGQSPKRLIYLVSKLDSGVPDRFTGSGSGTDFTLKISRVEAEDLGLYYCWQGTHFPWTFGGGTKLEIK

SEQ ID NO: 29 - protein, 117 aa, synthetic construct
QVQLQQPGAELVMPGASVKLSCKASAYTFTNYWMHWVKQRPGHGLEWIGEIDPSDSYTDYNQNFKAKATLTVDKSSSTAYMQLSSLTSEDSAVYYCARLMGRYFDVWGTGTTVTVSS

SEQ ID NO: 30 - protein, 107 aa, synthetic construct
DIVMTQSHKFMSTSVGDRVSITCKASQDVSAAVAWYQQKPGQSPKLLINSASYRYTGVPDRFTGSGSGTDFTFTISSVQAEDLAVYYCQQHYSTPLTFGAGTKLELR

SEQ ID NO: 31 - protein, 119 aa, synthetic construct
DVQLQESGPGLVKPSQSLSLTCSVTGYSITSGYYWNWIRQFPGNKLEWMGYISYDGGNNYNPSLKNRISITRDTSKNQFFLKLNSVTTEDTATYFCAREDYSNWYFDVWGTGTTVTVSS

SEQ ID NO: 32 - protein, 111 aa, synthetic construct
DIVLTQSPASLAVSLGQRATISCRASQSVSKSSYSYMHWYQQKPGQSPKLLIKYASILKSGVPARFSGSGSGTDFTLNIHPVEEEDTATYYCQHSWEIPWTFGGGTKLEIK

SEQ ID NO: 33 - protein, 119 aa, synthetic construct
EVQLQQSGAELVRPGSSVKMSCKTSGYTFTSYGINWVKQRPGQGLEWIGYIYIGNDYTEFNEKFKGKATLTSDTSSSTAYMQLSSLTSEDSAIYFCARFYSNSDPMDYWGHGTSVTVSS

SEQ ID NO: 34 - protein, 112 aa, synthetic construct
DVVMTQTPLTLSVSIGQPASISCKSSQSLLNSDGKTFLNWLLQRPGQSPKRLIYLVSKLDSGVPDRFTGSGSGTDFTLKISRVEAEDLGVYYCWQGTHFPLTFGAGTKLELK

SEQ ID NO: 35 - protein, 119 aa, unidentified
QVQLQQPGAELVKPGASVKLSCKASGYTFTNYWMQWVKQRPGQGLEWIGEIDPSDSYINYNQKFKGKATLTADTSSSTAYMQLSSLTYEDSAVYYCARPVTVPWYFDVWGTGTTVTVSS

SEQ ID NO: 36 - protein, 110 aa, synthetic construct
EIVLTQSPTTMAASPGEKITITCSATSSISSNYLHWYQQKPGFSPKLLIYRTSNLASGVPARFSGSGSGTSYSLTIGTMEAEDVATYYCQQGSAIPRIFTFGSGTKLEIK

SEQ ID NO: 37 - protein, 118 aa, synthetic construct
DVQLQESGPGLVKPSQSLSLTCSVTGYSITSGYDWNWIRQFPGNKLEWMGYISYDGKNNYNPSLRNRISITRDTSKNQFFLKLNSVTTEDTATYYCARRDLRGYFDVWGTGTTVTVSS

SEQ ID NO: 38 - protein, 107 aa, synthetic construct
DIVLTQSPATLSVTPGDRVSLSCRASQSISNYLHWYQQKSHESPRLLIKYASLSISGIPSRFSGSGSGTDFTLSINSVETEDFGVYFCQQSNSWPLTFGAGTKLELK

SEQ ID NO: 39 - protein, 114 aa, synthetic construct
QVQLQQSGAELVRPGASVTLSCKASGYTFPDYEIHWVKQTPVHGLEWIGAIDPETGGIGYNQKFTGKAMLTADKSSSTAYMELRSLTSEDSAVYFCTRNYGSRWGQGSTLTVSS

SEQ ID NO: 40 - protein, 112 aa, synthetic construct
DVVMTQTPLTLSVTIGQSASISCKSSQSLLESDGKTYLNWLLQRPGQSPKRLIYLVSKLDSGVPDRFTGSASGTDFTLKISRVEAEDLGVYYCWQGTHFPWTFGGGTKLEIK

SEQ ID NO: 41 - protein, 119 aa, synthetic construct
QVQLQQPGAELVVPGTSVKLSCKASGYTFTNYWMHWVKQRPGQGLEWIGEIDPSDNYANYNQEFQGKATLTVDKSSSTAYMQLSSLTSDDSAVYYCARHDGYFGALDYWGQGTSVTVSS

SEQ ID NO: 42 - protein, 110 aa, synthetic construct
EIVLTQSPTTMAASPGEKITITCSASSSISSNYLHWYQQKPGFSPKFLIYRTSNLASGVPARFSGSGSGTSYSLTIGTMEAEDVATYYCQQASSIPRMFTFGSGTKLEIK

SEQ ID NO: 43 - protein, 122 aa, synthetic construct
EVQLQQSGPVLVKPGASVKMSCKASGYTFTDYYMNWVKQRHGKSLEWIGISNPYNGGTSYNQKFKDKATLTVDKSSSTAYMELNSLTSEDSAVYYCAREGGTAQPTSGMDYWGQGTSVTVSS

SEQ ID NO: 44 - protein, 112 aa, synthetic construct
NIMMTQSPSSLAVSAGEKVTMSCKSSQSVLYSSNQKNYLAWYQQKPGQSPKLLIYWASTRESGVPDRFTGSGSGTDFTLTISSVQPEDPAVYYCHQYRSSYTFGGGTKLEIK

SEQ ID NO: 45 - protein, 117 aa, synthetic construct
QVQLQQPGAELVMPGASVKLSCKASGYTFTSYWMHWVKQRPGQGLEWIGEIDPSDSYTTYNQNFKGKATLTVDISTSTAYIQLSNLTSEDSAVYYCARLTGNYIHYWGQGTTLTVSS

SEQ ID NO: 46 - protein, 107 aa, synthetic construct
DIVMTQSHKFMSTSVGDRVSITCKASQDVSPAVAWYQQRPGQCPKLLIFSSSYRSTGVPDRFTGSGSGTDFTFTISSVQAEDLAVYYCQQHYSLPLTFGAGTKLELK

SEQ ID NO: 47 - protein, 119 aa, synthetic construct
QVQLQQPGAELVMPGASVKLSCKASGYTFTNYWMHWVKQRPGQGLEWIGEIDPSDYYANYNQKFKGKATLTVDKSSSTAYMQLSSLTSEDSAVYYCARSHYYANSYNYWGQGTTLTVSS

SEQ ID NO: 48 - protein, 110 aa, synthetic construct
EIELTQSPTTMAASPGEKITITCSASSSISSDYLHWYQQKPGFSPKLLIYRTSNLASGLPARFSGSGSGTSYSLTIGTMEAEDVATYYCQQGSSVPRMLTFGAGTKLELK

SEQ ID NO: 49 - protein, 119 aa, synthetic construct
EVQLQQSGAELVRPGSSVTMSCKTSGYTFTNYGINWVKQRPGQGLEWIGYIFIGNDYTEYNEKFKGKATLTSDTSSSTAYMQLSSLTSEDSAIYFCTRFYSNYYGMDPWGQGTSVTVSS

SEQ ID NO: 50 - protein, 112 aa, synthetic construct
DVVMTQTPLTLSVTIGQPASISCKSSQSLLHSDGKTYLNWLLQRPGQSPKRLIYLVSKLDSGVPDRFTGSGSGTDFTLKISRVEAEVLGVYYCWQGTHFPPTFGAGTKLEMK

SEQ ID NO: 51 - protein, 121 aa, synthetic construct
QVQLQQSGAELARPGASVKLSCKASGYTFTSYWMQWVKQRPGQGLEWIGAIYPGDGDSRYTQKFKGKATLTADKSSSTAYMQLSSLASEDSAVYYCARSTTTVLGNNFEYWGQGTTLTVSS

SEQ ID NO: 52 - protein, 106 aa, synthetic construct
QIVLTQSPAIMSALPGEKVTMTCSASSSVSSMHWYQQKSGTSPKRWIYDTSKLASGVPARFSGSGSGTSYSLTISSMEAEDAATYYCQQWSSNPWTFGGGTKLEIK

SEQ ID NO: 53 - protein, 122 aa, synthetic construct
QVQLQQSGPELVKPGASVKISCKASGYAFSSSWMNWLKQRPGQGLEWIGRIYPGDGDTNYNGKFKGKATLTADESSSTAYMQLSSLTSVDSAVYFCARGITTIITIAWFASWGQGTLVTVSA

SEQ ID NO: 54 - protein, 106 aa, synthetic construct
QIVLSQSPTILSASPGEKVTMTCRASSSVSYMHWYQQKPGSSPKPWIYATSNLASGVPPRFSGSGSGTSYSLTISRVGAEDAATYYCQQWSSDPWTFGGGTKLEIK

SEQ ID NO: 55 - protein, 122 aa, synthetic construct
QVQLQQSGPELVKPGASVKISCKASGYAFSSFWMNWVKQRPGEGLEWIGRIYPGDGDTNYNGKFKGKATLTADDSSSTAYMQLSSLTSVDSAVYFCAREVIAAVVTTDFDYWGQGTTLTVSS

SEQ ID NO: 56 - protein, 107 aa, synthetic construct
DIQMTQTTSSLSASLGDRVTISCRTSQDISNYLNWYLQKPDGTVKLLIYYTSGLHSGVPSRFSGSGSGTDYSLTISNLEPEDIATYFCQQGKTLPYTFGGGTKLEIK

SEQ ID NO: 57 - protein, 124 aa, synthetic construct
QVQLKQSGPGLVQPSQSLSITCTVSGFSLSTYGVHWVRQSPGRGLEWLGVIWIGGTTDYNAAFISRLTISKDNSRGQVFFKMDSLQANDTAIYYCARKGYYKYDGGYYYAMDYWGQGTSVTVSS

SEQ ID NO: 58 - protein, 107 aa, synthetic construct
DIQMTQSSSYLSVSLGGRVTITCKASDHINNWLAWYQQKPGNAPWLLISGATSLETGVPSRFSGSGSGKDYTLSISSLQTEDVATYYCQQYWSTPLTFGAGTKLELK

SEQ ID NO: 59 - protein, 122 aa, synthetic construct
QVQLQQSGPELVKPGASVKISCKASGYAFSSFWMNWVKQRPGQGLEWIGRIYPGDGDTNYNGKFKGKATLTADKSSTTAYMHLSSLTSVDSAVYFCTRSVITAVVDWYFDVWGAGTTVTVSS

SEQ ID NO: 60 - protein, 107 aa, synthetic construct
QIVLSQSPAILSASPGEKVTLTCRASSSVNFMHWYQQKPGSSPKPWIYATSNLASGAPARFSGSGSGTSYSLTISRVEAEDAAAYYCQQWSSYPIFTFGSGTKLEIK

SEQ ID NO: 61 - protein, 122 aa, synthetic construct
QVQLQQSGAELVRPGSSVKISCKGSGYAFSSYWMNWVKQRPGQGLEWIGQIYPGDGDTNYNGKFKGKATLTADKSSSTAYMQLSSLTSEDSAVYFCARAGFYYGSDSSMDYWGQGTSVTVSS

SEQ ID NO: 62 - protein, 111 aa, synthetic construct
DIVLTQSPASLAVSLGQRATISCRASESVDNFGISFMNWFQQKPGQPPKLLIYAASNQGSGVPARFSGSGSGTDFSLNIHPMEADDTAMYFCQQSKEVPYTFGGGTKLEIK

SEQ ID NO: 63 - protein, 116 aa, synthetic construct
EIQLQQSGPELVKPGASVKVSCKASGYAFTSYNMYWVKQSHGKSLEWIGYIDPYNGDTRYNQKFKGKATLTVDKSSSTAYMHLNSLTSEDSAVYYCTRSGTGRDYWGQGTTLTVSS

SEQ ID NO: 64 - protein, 106 aa, synthetic construct
QIVLTQSPAIMSASPGEKVTMTCSASSSISYMFWFQQKPGSSPRLLIYDTSSLASGVPVRFSGSGSGTSYTLTISRMEAEDAATYYCQQWSNYPYTFGGGTKLEMK

SEQ ID NO: 65 - protein, 120 aa, synthetic construct
QVQLQQSGAELARPGASVKLSCKASGYTFTSFWMQWLKQRPGQGLEWIGTIYPGDGDTRYTQKFKGKATLTADKSSNTAYMQLSSLASEDSAVYYCARGALSNYGGFAYWGQGTLVTVSA

SEQ ID NO: 66 - protein, 111 aa, synthetic construct
NIVLTQSPASLAVSLGQRATISCRASESVDSYGHSFMHWYQQKPGQPPKLLIYLASNLESGVPARFSGSGSRTDFTLTIDPVEADDAATYYCQQNNEDPWTFGGGTKLEIK

SEQ ID NO: 67 - protein, 123 aa, synthetic construct
QVQLQQSGAELVRPGTSVKVSCKASGYAFTNYLIEWVKQRPGQGLEWIGVINPGSGDTLYNEKFKGKATLTADKSSTTAYMQLSGLTSDVSAIYFCARSPPITTIVADYFDYWGQGTTLTVSS

SEQ ID NO: 68 - protein, 107 aa, synthetic construct
DIQMTQTTSSLSASLGDRVTISCRASQDISNYLNWYQQKPDGTVKLLIYYTSRLHSGVPSRFSGSGSGADYSLTISNLEQEDIATYFCQQGKTLPYTFGGGTKLEIK

SEQ ID NO: 69 - protein, 120 aa, synthetic construct
QMQLKESGPGLVAPSQSLSITCTVSGFSLTDYGVSWIRQPPGKGLEWLGVIWGSGSTFYNSALTSRLSISKDNSKSQVFLKMNSLQTADTAMYFCAKHHYYGGSFAMDYWGQGTSVTVSS

SEQ ID NO: 70 - protein, 107 aa, synthetic construct
DIQMTQASSSLSASLGDRVTISCKTSQDISNYLNWYQQKPDGTFKLLIHYTSRLHSGVPSRFSGSGSGSDYSLTISNLEREDIATYFCQQGNSLPYTFGGGTKLEMK

SEQ ID NO: 71 - protein, 121 aa, synthetic construct
DVQLRASGPGLVKPSQSLSLTCSVTGYSITSGYYWNWIRQFPGNKLEWMGCISYDGTNNYNPSLKNRISFTRDTSKNQFFLNLNSVTTEDSATYYCARRVYYRYDGVVDYWGQGTSVTVSS

SEQ ID NO: 72 - protein, 106 aa, synthetic construct
ENVLTQSPAIMSASPGEKVTMTCSASSSVSYIHWYQQKSSTAPKLWIYDTSKLASGVPGRFSGSRSRNSYSLTISSMEAEDVATYYCFQGSGYPLTFGSGTKLEIK

SEQ ID NO: 73 - protein, 121 aa, synthetic construct
QVQLQQPGAELVKPGASVKLSCKASGYTFTSYWMHWVKQRPGQGLEWIGEIDPSDSYSNYNQKFKGKATLTVDKSSSTAYMQLSSLTSEDSAVYYCARSNYGSSYGYFDVWGAGTTVTVSS

SEQ ID NO: 74 - protein, 105 aa, synthetic construct
QIVLTQSPAIMSASPGEKVTMTCSVSSSLSYMHWYQQKPGTSPKRWIYDTSKLASGVPARFSGSGSGTSYSLTISSMEAEDAATYYCHQRSSYPTFGGGTKLEIK

SEQ ID NO: 75 - protein, 120 aa, synthetic construct
QVQIQQSGAELARPGASVKLSCKASGYTFTNYWMQWIKQRPGQGLEWIGAIYPGDGDTRYTQKFKGKATLTADKSSSTAYMQLSSLASEDSAVYYCAREEVWSPYGMDYWGQGTSVTVSS

SEQ ID NO: 76 - protein, 106 aa, synthetic construct
QIVLTQSPAIMSASPGEKVTITCSASSSVSYMGWFQQKPGTSPKLWIYSTSNLASGVPARFSGSGSGTSYSLTISRMEAEDAATYYCQQRSIYPLTFGAGTKLELK

SEQ ID NO: 77 - protein, 125 aa, synthetic construct
QVTLKESGPGILQASQTLSLTCSFSGFSLSTFGIGVGWVRQPSGKGLEWLAHIWWNDNKFFNTTLKNRLTLSKDPSNNQVFLKIASVDTADTATYYCARSRSALITTGLYAMDYWGQGTSVTVSS

SEQ ID NO: 78 - protein, 107 aa, synthetic construct
DIQMTQTPSSLSASLGDRVTISCRSSQDISNYVNWYQQKPDGTVKVLINYTSRLHSGVPSRFSGSGSGTDYSLTISNLEQEDIASYFCQQGFTLPYTFGGGTKLEIK

SEQ ID NO: 79 - protein, 116 aa, synthetic construct
EIQLQQSGPELVKPGASVKVSCKASGYAFSAYNIYWVKQSHGKSLEWIGYIDPYNSGTTYNQKFRGKATLTVDKSSNTAYMHLSSLTSEDSAVYYCTRDGDAMDYWGQGTSVTVSS

SEQ ID NO: 80 - protein, 106 aa, synthetic construct
EILLTQSPAIIAASPGEKVTITCSASSGVIYMNWYQQKPGSSPKIWIYDVSTLASGVPARFSGSGSGTSFSFTINSMEAEDVATYYCQQRSSYPYTFGGGTKLEIK

SEQ ID NO: 81 - protein, 122 aa, synthetic construct
EVQLQQSGPELVKPGASVKMSCKASGYTFTSYVLHWVRQKPGQGLEWIGYFNPYNDGTEYNEKFKGKAILTSDKSSSTAYMELNSLTSEDSAVYYCVGGTYYYGSSYPFAYWGQGTLVTVST

SEQ ID NO: 82 - protein, 112 aa, synthetic construct
DVVMTQISLSLPVSLGDQASISCRSSQSLIHSNGNTYLQWYLQKPGQSPKLLIYKVSNRLSGVPDRFSGSGSGTDFTLKISRVEAEDLGVYFCSQSTHVPYTFGGGTKLEIK

SEQ ID NO: 83 - protein, 117 aa, synthetic construct
EVKLVESGGGLVQPGGSLKLSCAASGFTFSTYTMSWVRQTPEKRLEWVAFISSGGGHINYPDTVKGRFTISRDNAKNTLYLQMSSLKSEDTAMYYCARHSYWFFDVWGAGTTVTVSS

SEQ ID NO: 84 - protein, 107 aa, synthetic construct
DVQITQSPSYLAASPGETITINCRASKNIDTYLAWYQEKPGKTNKLLIYSGSTLQSGIPSRFRGGGSGTDFTLTICSLEPEDFAMYYCQQHNEYPLTFGAGTKLELK

SEQ ID NO: 85 - protein, 122 aa, synthetic construct
EVQLVESGGGLVKPGGSLKLSCAAAGFAFSSYDMSWVRQIPEKRLEWVAYISAGGGNTYFLDTVKGRFTISRDHAKNTLSLQMSSLKSEDTAMYFCVRHGDYYRYFYAMDYWGQGSSVTVSS

SEQ ID NO: 86 - protein, 107 aa, synthetic construct
DIVMTQSHKFMSTSVGDRVSITCKASQDVGTAVAWSQQKPGQSPKLLIYWASTRHTGVPDRFTGSGSGTDFTLTISNVQSEDLADYFCQQFVTYPYTFGGGTKLEIK

SEQ ID NO: 87 - protein, 121 aa, synthetic construct
QVQLQQPGAELVKPGASVKLSCKASGYTFTSYWMHWVKQRPGQGLEWIGEIDPSDSYTNYNQKFKGKATLTADKSSSTAYMQLSGLTSEDSAVYHCARGGDYDGYYVMDYWGQGTSVTVSS

SEQ ID NO: 88 - protein, 110 aa, synthetic construct
EIVLTQSPTTMAASPGEKITITCSASSSISSNYLHWYQQKPGFSPKLLIYRTSNLASGVPARFSGSGSGTSYSLTIGTMEADDVATYYCQQGSYIPRIFTFGSGTKLEIK

SEQ ID NO: 89 - protein, 119 aa, synthetic construct
EVQLQQSAPELVKPGASVKMSCKTSGYTFTENIIHWVKQTHGKSLEWIGGINPDNGGTSYHQKFKGRTTLTIDKSSSTAYMELRSLTSDDSAVFFCARQAPLYWYFDIWGAGTTVTVSS

SEQ ID NO: 90 - protein, 111 aa, synthetic construct
DIVLTQSPASLAVSLGQRATISCRASESVDSYGNSLMHWFQQKPGQPPRLLIYRASNLESGIPARFSGSGSRTDFTLTITPVEADDVATYYCQQSNEDPWTFGGGTKLEIK

SEQ ID NO: 91 - protein, 123 aa, synthetic construct
QVQLQQPGAELVRPGASVKLSCKASGYTFTSYWINWVKQRPGQGLEWIGNIHPSDSYTNYNQKFKDKATLTVDKSSSTAYMQFSSPTSEDSAVYYCTREDYYYGSNYDAMDYWGQGTSVTVSS

SEQ ID NO: 92 - protein, 107 aa, synthetic construct
DIVMTQSHKFMSTSVGDRVNITCKASQDVGSSVAWYQQKPGQSPKLLIYWASTRHAGVPDRFTGSGSGADFTLTISNVQSEDLADYFCQQYSTYPLTFGAGTKLELK

SEQ ID NO: 93 - protein, 120 aa, synthetic construct
QVQLKESGPGLVAPSQSLSITCTVSGFSLTDYGVSWIRQPPGKGLEWLGVIWGSETTFYNSALKSRLSISKDNSKSQLFLQMNSLQADDTAIYYCAKHHYYGGSFSMDYWGQGTSVTVSS

SEQ ID NO: 94 - protein, 107 aa, synthetic construct
DIQMTQTTSSLSASLGDRVTISCRASQDINNYLNWYQQKPDGTVKFLIYYTSRLHSGVPSRFSGSGSGTDYSLTISDLEQEDIATYFCQQGNTLPYTFGGGTKLEIK

SEQ ID NO: 95 - protein, 116 aa, synthetic construct
EIQLQQSGPELVKPGASVKVSCKASGYAFSAYNMYWVKQSHGKSLEWIGYIDPYNGGTNYNQKFKGKATLTVDKSSSTAYMHLNSLTSEDSAVYYCARDGYEVTYWGQGTLVTVSA

SEQ ID NO: 96 - protein, 106 aa, synthetic construct
QIVLTQSPALMSASLGEEITLTCSASSSVTYMHWSQQKSGTSPRLLIYSTSNLASGVPSRFSGSGSGTFYSLTISSVEAEDAADYYCHQWSSYPWTFGGGTKLEIK

SEQ ID NO: 97 - protein, 125 aa, synthetic construct
QVTLKESGPGILQPSQTLSLTCSFSGFSLSTFGLGVGWVRQPSGKGLEWLAHIWWDDDKYYNPALKSRVTVSKETSKNQVFFKIANVDTADSATYYCARLSRGLRRDVVYAMDHWGQGTSVTVSS

SEQ ID NO: 98 - protein, 107 aa, synthetic construct
DIQMTQTTSSLSASLGDRVTISCRASQDISNYLNWYQQKPDGSVKLLISYVSRLQSGVPSRFRGSGSGTDYSLTISNLDQEDIATYFCQQGIAFPYTFGGGTKLDIK

SEQ ID NO: 99 - protein, 122 aa, synthetic construct
DVQLQESGPGLVKPSQSQSLTCSVTGYSITSGYYWNWIRQFPGNKLEWMGYISYDGSNNYNPSLKNRISITRDTSKNQFFLKLNSVTTEDTVTYYCARAPLTGDRYWYFDVWGTGTTVTVSS

SEQ ID NO: 100 - protein, 111 aa, synthetic construct
DIVLTQSPASLAVSLGQRATISCRASQSVSTSSYSYMHWYQQKPGQTPKLLIKYASNLKSGVPARFSGSGSGTDFTLNIHPVEEEDTATYYCQHSWEIPPTFGGGTKLEIK

SEQ ID NO: 101 - protein, 121 aa, synthetic construct
QVTLKESGPGILQPSQTLSLTCSFSGFSLTTFGMGVGWIRQPSGKGLEWLTHIWWDDDKYYNPALKSRLTISKDTSKNQVFLRIANVDTADTATYYCARVITTGVPYFDYWGQGTTLTVSS

SEQ ID NO: 102 - protein, 108 aa, synthetic construct
ENVLTQSPAIMSASPGEKVTMTCRASSSVSSSYLYWYQQKSGASPKLWISSTSNLASGVPARFSGSGSGTSYSLTINSVEAEDAATYYCQQYSGYPWTFGGGTKLEIK

SEQ ID NO: 103 - protein, 117 aa, synthetic construct
QVQLHQPGAELVMPGASVTLSCKASGYTFTSYWMHWVKQRPGQGLEWIGEIDPSDSYTTYDQKFKGKATLTVDKFSSTAYMQFSSLTSEDSAVYYCARLTGNHLDYWGQGTTLTVSS

SEQ ID NO: 104 - protein, 107 aa, synthetic construct
DIVMTQSHKFMSSSVGDRVSITCKASQDVSPAVAWYQQKPGQSPKLLIYSTSYRNTGVPDRFTGSGSGTDFTFTISSVQAEDLAVYYCQQHYSIPLTFGAGTKLELK

SEQ ID NO: 105 - protein, 120 aa, synthetic construct
DVQLQESGPGLVKPSQSLSLTCSVTDYSITSGYYWTWIRQFPGNKLEWMGYISYDGSTNYNPSLKNRFSITRDTSKNQFFLKLNSVIIEDTATYYCARDRMSTTWYFDVWGTGTTVTVSS

SEQ ID NO: 106 - protein, 111 aa, synthetic construct
DIVLTQSPASLAVSLGQRATISCRASESVDNYGISFMHWYQQKPGQPPKLLIYRASKTESGIPARFSGSGSRTDFTLTINPVETDDVATYYCQQSNKYPRTFGGGTKVEIK

SEQ ID NO: 107 - protein, 123 aa, synthetic construct
EVQLVESGGDLVKPGGSLKLSCAASGFTFSSYGMSWVRQTPDKRLEWVATISHGGSYTHYPDSVKGRFTISRDNAKNTLYLQMNSLKSEDTAMYYCVRLPITTVEAPYFFDYWGQGTTLTVSS

SEQ ID NO: 108 - protein, 106 aa, synthetic construct
DIQMTQTTSSLSASLGDRVTISCRASQDIRNYLNWYQQKPDGTVKLLIYYTSILHSGVPSRFSGSGSGTDYSLTINNLEQEDVATYFCQQGNTLYTFGGGTEVELR

SEQ ID NO: 109 - protein, 122 aa, synthetic construct
QVQLQQSGAELVKPGASVKISCKASGYAFSSYWMNWVKQRPGKGLEWIGQIYPGDGDTNYNGKFKGKATLTADKSSSTGYMQLSSLTSEDSAVYFCARSRITSVVDWYFDVWGTGTTVTVSS

SEQ ID NO: 110 - protein, 106 aa, synthetic construct
QIVLSQSPAILSASPGEKVTMTCRASSSVSYMHWYQQKPGSSPKPWIYATSNLASGVPARFSGSGSGTSYSLTISRVEAEDAATYYCQQWSSNPPTFGAGTKLELK

SEQ ID NO: 111 - protein, 121 aa, synthetic construct
QVQLQQPGAELVKPGASVKLSCKASGYTFTSYWMQWVKQRPGQGLEWIGEIDPSDSYTNYNQKFKGKASLTVDTSSSTAYMQLSSLTSEDSAVYYCARWGLLRNYYVMDYWGQGTSVTVSS

SEQ ID NO: 112 - protein, 110 aa, synthetic construct
EIVLTQSPTTMAASPGEKITITCSASSSISSNYLHWYQQKPGFSPKLLIYRTSNLASGVPARFSGSGSGTSYSLTIGTMEAEDVATYYCQQGSSIPRMLTFGAGTKLELK

SEQ ID NO: 113 - protein, 118 aa, synthetic construct
DVQLQESGPGLVKPSQSLSLTCSVTGYSITSGYYWIWIRQFPGNKLEWMGYISYDASNKYKPSLKNRISITRDTSKNQFFLKLNSVTAEDTATYFCAREDLRGYFDVWGTGTSVTVSS

SEQ ID NO: 114 - protein, 111 aa, synthetic construct
DIVLTQSPASLAVSLGRRATISCRASQSVSTSGFSYMHWYQQKPGQPPNLLIKYASILQSGVPARFSGSGSGTDFILNIHPVEDVDTATYYCQHSWGIPFTFGSGTKLEIK

SEQ ID NO: 115 - protein, 5 aa, synthetic construct
DYVMH

SEQ ID NO: 116 - protein, 17 aa, synthetic construct
YFNPYNDGTNYNEKFKV

SEQ ID NO: 117 - protein, 11 aa, synthetic construct
GVYYYGRDFDY

SEQ ID NO: 118 - protein, 16 aa, synthetic construct
RSSQSLENSNGNSYLN

SEQ ID NO: 119 - protein, 7 aa, synthetic construct
RVSNRFS

SEQ ID NO: 120 - protein, 9 aa, synthetic construct
LQITHVPWT

SEQ ID NO: 121 - protein, 5 aa, synthetic construct
DYGVS

SEQ ID NO: 122 - protein, 16 aa, synthetic construct
VIWGSGDTYYNSVLES

SEQ ID NO: 123 - protein, 12 aa, synthetic construct
HSYYGGSFAMDY

SEQ ID NO: 124 - protein, 11 aa, synthetic construct
RASQDISNYLN

SEQ ID NO: 125 - protein, 7 aa, synthetic construct
YTSRLHS

SEQ ID NO: 126 - protein, 9 aa, synthetic construct
QQGKTLPWT

SEQ ID NO: 127 - protein, 6 aa, synthetic construct
SGYYWN

SEQ ID NO: 128 - protein, 16 aa, synthetic construct
HISYDGNNNYNPSLKN

SEQ ID NO: 129 - protein, 10 aa, synthetic construct
ENYSNYYFDY

SEQ ID NO: 130 - protein, 15 aa, synthetic construct
RASQSVSKSSYTYIH

SEQ ID NO: 131 - protein, 7 aa, synthetic construct
YASILQS

SEQ ID NO: 132 - protein, 9 aa, synthetic construct
QHSWEIPYT

SEQ ID NO: 133 - protein, 5 aa, synthetic construct
GSWMN

SEQ ID NO: 134 - protein, 17 aa, synthetic construct
RIYPGDGDTYYNGKFKD

SEQ ID NO: 135 - protein, 9 aa, synthetic construct
LRYRYVMDY

SEQ ID NO: 136 - protein, 15 aa, synthetic construct
RASESVSIHGSHLMH

SEQ ID NO: 137 - protein, 7 aa, synthetic construct
AASNLES

SEQ ID NO: 138 - protein, 9 aa, synthetic construct
QQGIKDPYT

SEQ ID NO: 139 - protein, 6 aa, synthetic construct
SGYYWN

SEQ ID NO: 140 - protein, 16 aa, synthetic construct
YISYDGSNNYNPSLKN

SEQ ID NO: 141 - protein, 11 aa, synthetic construct
RKLTGGPYFDY

SEQ ID NO: 142 - protein, 15 aa, synthetic construct
RASESVSFHGFHIMH

SEQ ID NO: 143 - protein, 7 aa, synthetic construct
AASHLVS

SEQ ID NO: 144 - protein, 9 aa, synthetic construct
QQSVEDPWT

SEQ ID NO: 145 - protein, 5 aa, synthetic construct
DYNMN

SEQ ID NO: 146 - protein, 17 aa, synthetic construct
IINPNFGSTSYNQKFKG

SEQ ID NO: 147 - protein, 11 aa, synthetic construct
SEYYGSSGFAY

SEQ ID NO: 148 - protein, 16 aa, synthetic construct
RSSQSLVNSYGNTYLS

SEQ ID NO: 149 - protein, 7 aa, synthetic construct
GISNRFS

SEQ ID NO: 150 - protein, 9 aa, synthetic construct
LQGTHQPWT

SEQ ID NO: 151 - protein, 5 aa, synthetic construct
GSWMN

SEQ ID NO: 152 - protein, 17 aa, synthetic construct
RIYPGDGDTYYSGKFKD

SEQ ID NO: 153 - protein, 9 aa, synthetic construct
LRSRYVMDY

SEQ ID NO: 154 - protein, 15 aa, synthetic construct
RASESVSIHGTHLMH

SEQ ID NO: 155 - protein, 7 aa, synthetic construct
AASNLES

SEQ ID NO: 156 - protein, 9 aa, synthetic construct
QQGIDDPYT

SEQ ID NO: 157 - protein, 5 aa, synthetic construct
DYHIN

SEQ ID NO: 158 - protein, 17 aa, synthetic construct
DINPNNGGTTYNQKFKD

SEQ ID NO: 159 - protein, 12 aa, synthetic construct
FITTVVAWYFDV

SEQ ID NO: 160 - protein, 11 aa, synthetic construct
RASENIYSNLA

SEQ ID NO: 161 - protein, 7 aa, synthetic construct
AATNLAD

SEQ ID NO: 162 - protein, 9 aa, synthetic construct
QRFWDTPRT

SEQ ID NO: 163 - protein, 5 aa, synthetic construct
DYEMH

SEQ ID NO: 164 - protein, 17 aa, synthetic construct
GIAPETGLTTYNQKFED

SEQ ID NO: 165 - protein, 5 aa, synthetic construct
NNYGL

SEQ ID NO: 166 - protein, 16 aa, synthetic construct
KSSQSLLDSNGKTYLN

SEQ ID NO: 167 - protein, 7 aa, synthetic construct
LVSKLDS

SEQ ID NO: 168 - protein, 9 aa, unidentified
WQGTHFPWT

SEQ ID NO: 169 - protein, 5 aa, synthetic construct
DYNMN

SEQ ID NO: 170 - protein, 16 aa, synthetic construct
TINPNYITSYNQKFKG

SEQ ID NO: 171 - protein, 5 aa, synthetic construct
DYKGY

SEQ ID NO: 172 - protein, 16 aa, synthetic construct
KSSQNLLDSDGKTYLN

SEQ ID NO: 173 - protein, 7 aa, synthetic construct
LVSKLDS

SEQ ID NO: 174 - protein, 9 aa, synthetic construct
WQGTHFPWT

SEQ ID NO: 175 - protein, 5 aa, synthetic construct
NYWMH

SEQ ID NO: 176 - protein, 17 aa, synthetic construct
EIDPSDSYTDYNQNFKA

SEQ ID NO: 177 - protein, 8 aa, synthetic construct
LMGRYFDV

SEQ ID NO: 178 - protein, 11 aa, synthetic construct
KASQDVSAAVA

SEQ ID NO: 179 - protein, 7 aa, synthetic construct
SASYRYT

SEQ ID NO: 180 - protein, 9 aa, synthetic construct
QQHYSTPLT

SEQ ID NO: 181 - protein, 6 aa, synthetic construct
SGYYWN

SEQ ID NO: 182 - protein, 16 aa, synthetic construct
YISYDGGNNYNPSLKN

SEQ ID NO: 183 - protein, 10 aa, synthetic construct
EDYSNWYFDV

SEQ ID NO: 184 - protein, 15 aa, synthetic construct
RASQSVSKSSYSYMH

SEQ ID NO: 185 - protein, 7 aa, synthetic construct
YASILKS

SEQ ID NO: 186 - protein, 9 aa, synthetic construct
QHSWEIPWT

SEQ ID NO: 187 - protein, 5 aa, synthetic construct
SYGIN

SEQ ID NO: 188 - protein, 17 aa, synthetic construct
YIYIGNDYTEFNEKFKG

SEQ ID NO: 189 - protein, 10 aa, synthetic construct
FYSNSDPMDY

SEQ ID NO: 190 - protein, 16 aa, synthetic construct
KSSQSLLNSDGKTFLN

SEQ ID NO: 191 - protein, 7 aa, synthetic construct
LVSKLDS

SEQ ID NO: 192 - protein, 9 aa, synthetic construct
WQGTHFPLT

SEQ ID NO: 193 - protein, 5 aa, synthetic construct
NYWMQ

SEQ ID NO: 194 - protein, 17 aa, synthetic construct
EIDPSDSYINYNQKFKG

SEQ ID NO: 195 - protein, 10 aa, synthetic construct
PVTVPWYFDV

SEQ ID NO: 196 - protein, 12 aa, synthetic construct
SATSSISSNYLH

SEQ ID NO: 197 - protein, 7 aa, synthetic construct
RTSNLAS

SEQ ID NO: 198 - protein, 11 aa, synthetic construct
QQGSAIPRIFT

SEQ ID NO: 199 - protein, 6 aa, synthetic construct
SGYDWN

SEQ ID NO: 200 - protein, 16 aa, synthetic construct
YISYDGKNNYNPSLRN

SEQ ID NO: 201 - protein, 9 aa, synthetic construct
RDLRGYFDV

SEQ ID NO: 202 - protein, 11 aa, synthetic construct
RASQSISNYLH

SEQ ID NO: 203 - protein, 7 aa, synthetic construct
YASLSIS

SEQ ID NO: 204 - protein, 9 aa, synthetic construct
QQSNSWPLT

SEQ ID NO: 205 - protein, 5 aa, synthetic construct
DYEIH

SEQ ID NO: 206 - protein, 17 aa, synthetic construct
AIDPETGGIGYNQKFTG

SEQ ID NO: 207 - protein, 5 aa, synthetic construct
NYGSR

SEQ ID NO: 208 - protein, 16 aa, synthetic construct
KSSQSLLESDGKTYLN

SEQ ID NO: 209 - protein, 7 aa, synthetic construct
LVSKLDS

SEQ ID NO: 210 - protein, 9 aa, synthetic construct
WQGTHFPWT

SEQ ID NO: 211 - protein, 5 aa, synthetic construct
NYWMH

SEQ ID NO: 212 - protein, 17 aa, synthetic construct
EIDPSDNYANYNQEFQG

SEQ ID NO: 213 - protein, 10 aa, synthetic construct
HDGYFGALDY

SEQ ID NO: 214 - protein, 12 aa, synthetic construct
SASSSISSNYLH

SEQ ID NO: 215 - protein, 7 aa, synthetic construct
RTSNLAS

SEQ ID NO: 216 - protein, 11 aa, synthetic construct
QQASSIPRMFT

SEQ ID NO: 217 - protein, 5 aa, synthetic construct
DYYMN

SEQ ID NO: 218 - protein, 17 aa, synthetic construct
ISNPYNGGTSYNQKFKD

SEQ ID NO: 219 - protein, 13 aa, synthetic construct
EGGTAQPTSGMDY

SEQ ID NO: 220 - protein, 17 aa, synthetic construct
KSSQSVLYSSNQKNYLA

SEQ ID NO: 221 - protein, 7 aa, synthetic construct
WASTRES

SEQ ID NO: 222 - protein, 8 aa, synthetic construct
HQYRSSYT

SEQ ID NO: 223 - protein, 5 aa, synthetic construct
SYWMH

SEQ ID NO: 224 - protein, 17 aa, synthetic construct
EIDPSDSYTTYNQNFKG

SEQ ID NO: 225 - protein, 8 aa, synthetic construct
LTGNYIHY

SEQ ID NO: 226 - protein, 11 aa, synthetic construct
KASQDVSPAVA

SEQ ID NO: 227 - protein, 7 aa, synthetic construct
SSSYRST

SEQ ID NO: 228 - protein, 9 aa, synthetic construct
QQHYSLPLT

SEQ ID NO: 229 - protein, 5 aa, synthetic construct
NYWMH

SEQ ID NO: 230 - protein, 17 aa, synthetic construct
EIDPSDYYANYNQKFKG

SEQ ID NO: 231 - protein, 10 aa, synthetic construct
SHYYANSYNY

SEQ ID NO: 232 - protein, 12 aa, synthetic construct
SASSSISSDYLH

SEQ ID NO: 233 - protein, 7 aa, synthetic construct
RTSNLAS

SEQ ID NO: 234 - protein, 11 aa, synthetic construct
QQGSSVPRMLT

SEQ ID NO: 235 - protein, 5 aa, synthetic construct
NYGIN

SEQ ID NO: 236 - protein, 17 aa, synthetic construct
YIFIGNDYTEYNEKFKG

SEQ ID NO: 237 - protein, 10 aa, synthetic construct
FYSNYYGMDP

SEQ ID NO: 238 - protein, 16 aa, synthetic construct
KSSQSLLHSDGKTYLN

SEQ ID NO: 239 - protein, 7 aa, synthetic construct
LVSKLDS

SEQ ID NO: 240 - protein, 9 aa, synthetic construct
WQGTHFPPT

SEQ ID NO: 241 - protein, 5 aa, synthetic construct
SYWMQ

SEQ ID NO: 242 - protein, 17 aa, synthetic construct
AIYPGDGDSRYTQKFKG

SEQ ID NO: 243 - protein, 12 aa, synthetic construct
STTTVLGNNFEY

SEQ ID NO: 244 - protein, 10 aa, synthetic construct
SASSSVSSMH

SEQ ID NO: 245 - protein, 10 aa, synthetic construct
SASSSVSSMH

SEQ ID NO: 246 - protein, 9 aa, synthetic construct
QQWSSNPWT

SEQ ID NO: 247 - protein, 5 aa, synthetic construct
SSWMN

SEQ ID NO: 248 - protein, 17 aa, synthetic construct
RIYPGDGDTNYNGKFKG

SEQ ID NO: 249 - protein, 13 aa, synthetic construct
GITTIITIAWFAS

SEQ ID NO: 250 - protein, 10 aa, synthetic construct
RASSSVSYMH

SEQ ID NO: 251 - protein, 7 aa, synthetic construct
ATSNLAS

SEQ ID NO: 252 - protein, 9 aa, synthetic construct
QQWSSDPWT

SEQ ID NO: 253 - protein, 5 aa, synthetic construct
SFWMN

SEQ ID NO: 254 - protein, 17 aa, synthetic construct
RIYPGDGDTNYNGKFKG

SEQ ID NO: 255 - protein, 13 aa, synthetic construct
EVIAAVVTTDFDY

SEQ ID NO: 256 - protein, 11 aa, synthetic construct
RTSQDISNYLN

SEQ ID NO: 257 - protein, 7 aa, synthetic construct
YTSGLHS

SEQ ID NO: 258 - protein, 9 aa, synthetic construct
QQGKTLPYT

SEQ ID NO: 259 - protein, 5 aa, synthetic construct
TYGVH

SEQ ID NO: 260 - protein, 16 aa, synthetic construct
VIWIGGTTDYNAAFIS

SEQ ID NO: 261 - protein, 16 aa, synthetic construct
KGYYKYDGGYYYAMDY

SEQ ID NO: 262 - protein, 11 aa, synthetic construct
KASDHINNWLA

SEQ ID NO: 263 - protein, 7 aa, synthetic construct
GATSLET

SEQ ID NO: 264 - protein, 9 aa, synthetic construct
QQYWSTPLT

SEQ ID NO: 265 - protein, 5 aa, synthetic construct
SFWMN

SEQ ID NO: 266 - protein, 17 aa, synthetic construct
RIYPGDGDTNYNGKFKG

SEQ ID NO: 267 - protein, 13 aa, synthetic construct
SVITAVVDWYFDV

SEQ ID NO: 268 - protein, 10 aa, synthetic construct
RASSSVNFMH

SEQ ID NO: 269 - protein, 7 aa, synthetic construct
ATSNLAS

SEQ ID NO: 270 - protein, 10 aa, synthetic construct
QQWSSYPIFT

SEQ ID NO: 271 - protein, 5 aa, synthetic construct
SYWMN

SEQ ID NO: 272 - protein, 17 aa, synthetic construct
QIYPGDGDTNYNGKFKG

SEQ ID NO: 273 - protein, 13 aa, synthetic construct
AGFYYGSDSSMDY

SEQ ID NO: 274 - protein, 15 aa, synthetic construct
RASESVDNFGISFMN

SEQ ID NO: 275 - protein, 7 aa, synthetic construct
AASNQGS

SEQ ID NO: 276 - protein, 9 aa, synthetic construct
QQSKEVPYT

SEQ ID NO: 277 - protein, 5 aa, synthetic construct
SYNMY

SEQ ID NO: 278 - protein, 17 aa, synthetic construct
YIDPYNGDTRYNQKFKG

SEQ ID NO: 279 - protein, 7 aa, synthetic construct
SGTGRDY

SEQ ID NO: 280 - protein, 10 aa, synthetic construct
SASSSISYMF

SEQ ID NO: 281 - protein, 7 aa, synthetic construct
DTSSLAS

SEQ ID NO: 282 - protein, 9 aa, synthetic construct
QQWSNYPYT

SEQ ID NO: 283 - protein, 5 aa, synthetic construct
SFWMQ

SEQ ID NO: 284 - protein, 17 aa, synthetic construct
TIYPGDGDTRYTQKFKG

SEQ ID NO: 285 - protein, 11 aa, synthetic construct
GALSNYGGFAY

SEQ ID NO: 286 - protein, 15 aa, synthetic construct
RASESVDSYGHSFMH

SEQ ID NO: 287 - protein, 7 aa, synthetic construct
LASNLES

SEQ ID NO: 288 - protein, 9 aa, synthetic construct
QQNNEDPWT

SEQ ID NO: 289 - protein, 5 aa, synthetic construct
NYLIE

SEQ ID NO: 290 - protein, 17 aa, synthetic construct
VINPGSGDTLYNEKFKG

SEQ ID NO: 291 - protein, 14 aa, synthetic construct
SPPITTIVADYFDY

SEQ ID NO: 292 - protein, 11 aa, synthetic construct
RASQDISNYLN

SEQ ID NO: 293 - protein, 7 aa, synthetic construct
YTSRLHS

SEQ ID NO: 294 - protein, 9 aa, synthetic construct
QQGKTLPYT

SEQ ID NO: 295 - protein, 5 aa, synthetic construct
DYGVS

SEQ ID NO: 296 - protein, 16 aa, synthetic construct
VIWGSGSTFYNSALTS

SEQ ID NO: 297 - protein, 12 aa, synthetic construct
HHYYGGSFAMDY

SEQ ID NO: 298 - protein, 11 aa, synthetic construct
KTSQDISNYLN

SEQ ID NO: 299 - protein, 7 aa, synthetic construct
YTSRLHS

SEQ ID NO: 300 - protein, 9 aa, synthetic construct
QQGNSLPYT

SEQ ID NO: 301 - protein, 6 aa, synthetic construct
SGYYWN

SEQ ID NO: 302 - protein, 16 aa, synthetic construct
CISYDGTNNYNPSLKN

SEQ ID NO: 303 - protein, 12 aa, synthetic construct
RVYYRYDGVVDY

SEQ ID NO: 304 - protein, 10 aa, synthetic construct
SASSSVSYIH

SEQ ID NO: 305 - protein, 7 aa, synthetic construct
DTSKLAS

SEQ ID NO: 306 - protein, 9 aa, synthetic construct
FQGSGYPLT

SEQ ID NO: 307 - protein, 5 aa, synthetic construct
SYWMH

SEQ ID NO: 308 - protein, 17 aa, synthetic construct
EIDPSDSYSNYNQKFKG

SEQ ID NO: 309 - protein, 12 aa, synthetic construct
SNYGSSYGYFDV

SEQ ID NO: 310 - protein, 10 aa, synthetic construct
SVSSSLSYMH

SEQ ID NO: 311 - protein, 7 aa, synthetic construct
DTSKLAS

SEQ ID NO: 312 - protein, 8 aa, synthetic construct
HQRSSYPT

SEQ ID NO: 313 - protein, 5 aa, synthetic construct
NYWMQ

SEQ ID NO: 314 - protein, 17 aa, synthetic construct
AIYPGDGDTRYTQKFKG

SEQ ID NO: 315 - protein, 11 aa, synthetic construct
EEVWSPYGMDY

SEQ ID NO: 316 - protein, 10 aa, synthetic construct
SASSSVSYMG

SEQ ID NO: 317 - protein, 7 aa, synthetic construct
STSNLAS

SEQ ID NO: 318 - protein, 9 aa, synthetic construct
QQRSIYPLT

SEQ ID NO: 319 - protein, 7 aa, synthetic construct
TFGIGVG

SEQ ID NO: 320 - protein, 16 aa, synthetic construct
HIWWNDNKFFNTTLKN

SEQ ID NO: 321 - protein, 15 aa, synthetic construct
SRSALITTGLYAMDY

SEQ ID NO: 322 - protein, 11 aa, synthetic construct
RSSQDISNYVN

SEQ ID NO: 323 - protein, 7 aa, synthetic construct
YTSRLHS

SEQ ID NO: 324 - protein, 9 aa, synthetic construct
QQGFTLPYT

SEQ ID NO: 325 - protein, 5 aa, synthetic construct
AYNIY

SEQ ID NO: 326 - protein, 17 aa, synthetic construct
YIDPYNSGTTYNQKFRG

SEQ ID NO: 327 - protein, 7 aa, synthetic construct
DGDAMDY

SEQ ID NO: 328 - protein, 10 aa, synthetic construct
SASSGVIYMN

SEQ ID NO: 329 - protein, 7 aa, synthetic construct
DVSTLAS

SEQ ID NO: 330 - protein, 9 aa, synthetic construct
QQRSSYPYT

SEQ ID NO: 331 - protein, 5 aa, synthetic construct
SYVLH

SEQ ID NO: 332 - protein, 17 aa, synthetic construct
YFNPYNDGTEYNEKFKG

SEQ ID NO: 333 - protein, 13 aa, synthetic construct
GTYYYGSSYPFAY

SEQ ID NO: 334 - protein, 16 aa, synthetic construct
RSSQSLIHSNGNTYLQ

SEQ ID NO: 335 - protein, 7 aa, synthetic construct
KVSNRLS

SEQ ID NO: 336 - protein, 9 aa, synthetic construct
SQSTHVPYT

SEQ ID NO: 337 - protein, 5 aa, synthetic construct
TYTMS

SEQ ID NO: 338 - protein, 17 aa, synthetic construct
FISSGGGHINYPDTVKG

SEQ ID NO: 339 - protein, 8 aa, synthetic construct
HSYWFFDV

SEQ ID NO: 340 - protein, 11 aa, synthetic construct
RASKNIDTYLA

SEQ ID NO: 341 - protein, 7 aa, synthetic construct
SGSTLQS

SEQ ID NO: 342 - protein, 9 aa, synthetic construct
QQHNEYPLT

SEQ ID NO: 343 - protein, 5 aa, synthetic construct
SYDMS

SEQ ID NO: 344 - protein, 17 aa, synthetic construct
YISAGGGNTYFLDTVKG

SEQ ID NO: 345 - protein, 13 aa, synthetic construct
HGDYYRYFYAMDY

SEQ ID NO: 346 - protein, 11 aa, synthetic construct
KASQDVGTAVA

SEQ ID NO: 347 - protein, 7 aa, synthetic construct
WASTRHT

SEQ ID NO: 348 - protein, 9 aa, synthetic construct
QQFVTYPYT

SEQ ID NO: 349 - protein, 5 aa, synthetic construct
SYWMH

SEQ ID NO: 350 - protein, 17 aa, synthetic construct
EIDPSDSYTNYNQKFKG

SEQ ID NO: 351 - protein, 12 aa, synthetic construct
GGDYDGYYVMDY

SEQ ID NO: 352 - protein, 12 aa, synthetic construct
SASSSISSNYLH

SEQ ID NO: 353 - protein, 7 aa, synthetic construct
RTSNLAS

SEQ ID NO: 354 - protein, 11 aa, synthetic construct
QQGSYIPRIFT

SEQ ID NO: 355 - protein, 5 aa, synthetic construct
ENIIH

SEQ ID NO: 356 - protein, 17 aa, synthetic construct
GINPDNGGTSYHQKFKG

SEQ ID NO: 357 - protein, 10 aa, synthetic construct
QAPLYWYFDI

SEQ ID NO: 358 - protein, 15 aa, synthetic construct
RASESVDSYGNSLMH

SEQ ID NO: 359 - protein, 7 aa, synthetic construct
RASNLES

SEQ ID NO: 360 - protein, 9 aa, synthetic construct
QQSNEDPWT

SEQ ID NO: 361 - protein, 5 aa, synthetic construct
SYWIN

SEQ ID NO: 362 - protein, 17 aa, synthetic construct
NIHPSDSYTNYNQKFKD

SEQ ID NO: 363 - protein, 14 aa, synthetic construct
EDYYYGSNYDAMDY

SEQ ID NO: 364 - protein, 11 aa, synthetic construct
KASQDVGSSVA

SEQ ID NO: 365 - protein, 7 aa, synthetic construct
WASTRHA

SEQ ID NO: 366 - protein, 9 aa, synthetic construct
QQYSTYPLT

SEQ ID NO: 367 - protein, 5 aa, synthetic construct
DYGVS

SEQ ID NO: 368 - protein, 16 aa, synthetic construct
VIWGSETTFYNSALKS

SEQ ID NO: 369 - protein, 12 aa, synthetic construct
HHYYGGSFSMDY

SEQ ID NO: 370 - protein, 11 aa, synthetic construct
RASQDINNYLN

SEQ ID NO: 371 - protein, 7 aa, synthetic construct
YTSRLHS

SEQ ID NO: 372 - protein, 9 aa, synthetic construct
QQGNTLPYT

SEQ ID NO: 373 - protein, 5 aa, synthetic construct
AYNMY

SEQ ID NO: 374 - protein, 17 aa, synthetic construct
YIDPYNGGTNYNQKFKG

SEQ ID NO: 375 - protein, 7 aa, synthetic construct
DGYEVTY

SEQ ID NO: 376 - protein, 10 aa, synthetic construct
SASSSVTYMH

SEQ ID NO: 377 - protein, 7 aa, synthetic construct
STSNLAS

SEQ ID NO: 378 - protein, 9 aa, synthetic construct
HQWSSYPWT

SEQ ID NO: 379 - protein, 7 aa, synthetic construct
TFGLGVG

SEQ ID NO: 380 - protein, 16 aa, synthetic construct
HIWWDDDKYYNPALKS

SEQ ID NO: 381 - protein, 15 aa, synthetic construct
LSRGLRRDVVYAMDH

SEQ ID NO: 382 - protein, 11 aa, synthetic construct
RASQDISNYLN

SEQ ID NO: 383 - protein, 7 aa, synthetic construct
YVSRLQS

SEQ ID NO: 384 - protein, 9 aa, synthetic construct
QQGIAFPYT

SEQ ID NO: 385 - protein, 6 aa, synthetic construct
SGYYWN

SEQ ID NO: 386 - protein, 16 aa, synthetic construct
YISYDGSNNYNPSLKN

SEQ ID NO: 387 - protein, 13 aa, synthetic construct
APLTGDRYWYFDV

SEQ ID NO: 388 - protein, 15 aa, synthetic construct
RASQSVSTSSYSYMH

SEQ ID NO: 389 - protein, 7 aa, synthetic construct
YASNLKS

SEQ ID NO: 390 - protein, 9 aa, synthetic construct
QHSWEIPPT

SEQ ID NO: 391 - protein, 7 aa, synthetic construct
TFGMGVG

SEQ ID NO: 392 - protein, 16 aa, synthetic construct
HIWWDDDKYYNPALKS

SEQ ID NO: 393 - protein, 11 aa, synthetic construct
VITTGVPYFDY

SEQ ID NO: 394 - protein, 12 aa, synthetic construct
RASSSVSSSYLY

SEQ ID NO: 395 - protein, 7 aa, synthetic construct
STSNLAS

SEQ ID NO: 396 - protein, 7 aa, synthetic construct
STSNLAS

SEQ ID NO: 397 - protein, 5 aa, synthetic construct
SYWMH

SEQ ID NO: 398 - protein, 5 aa, synthetic construct
SYWMH

SEQ ID NO: 399 - protein, 8 aa, synthetic construct
LTGNHLDY

SEQ ID NO: 400 - protein, 11 aa, synthetic construct
KASQDVSPAVA

SEQ ID NO: 401 - protein, 7 aa, synthetic construct
STSYRNT

SEQ ID NO: 402 - protein, 9 aa, synthetic construct
QQHYSIPLT

SEQ ID NO: 403 - protein, 6 aa, synthetic construct
SGYYWT

SEQ ID NO: 404 - protein, 16 aa, synthetic construct
YISYDGSTNYNPSLKN

SEQ ID NO: 405 - protein, 11 aa, synthetic construct
DRMSTTWYFDV

SEQ ID NO: 406 - protein, 15 aa, synthetic construct
RASESVDNYGISFMH

SEQ ID NO: 407 - protein, 7 aa, synthetic construct
RASKTES

SEQ ID NO: 408 - protein, 9 aa, synthetic construct
QQSNKYPRT

SEQ ID NO: 409 - protein, 5 aa, synthetic construct
SYGMS

SEQ ID NO: 410 - protein, 17 aa, synthetic construct
TISHGGSYTHYPDSVKG

SEQ ID NO: 411 - protein, 14 aa, synthetic construct
LPITTVEAPYFFDY

SEQ ID NO: 412 - protein, 11 aa, synthetic construct
RASQDIRNYLN

SEQ ID NO: 413 - protein, 7 aa, synthetic construct
YTSILHS

SEQ ID NO: 414 - protein, 8 aa, synthetic construct
QQGNTLYT

SEQ ID NO: 415 - protein, 5 aa, synthetic construct
SYWMN

SEQ ID NO: 416 - protein, 17 aa, synthetic construct
QIYPGDGDTNYNGKFKG

SEQ ID NO: 417 - protein, 13 aa, synthetic construct
SRITSVVDWYFDV

SEQ ID NO: 418 - protein, 10 aa, synthetic construct
RASSSVSYMH

SEQ ID NO: 419 - protein, 7 aa, synthetic construct
ATSNLAS

SEQ ID NO: 420 - protein, 9 aa, synthetic construct
QQWSSNPPT

SEQ ID NO: 421 - protein, 5 aa, synthetic construct
SYWMQ

SEQ ID NO: 422 - protein, 17 aa, synthetic construct
EIDPSDSYTNYNQKFKG

SEQ ID NO: 423 - protein, 12 aa, synthetic construct
WGLLRNYYVMDY

SEQ ID NO: 424 - protein, 12 aa, synthetic construct
SASSSISSNYLH

SEQ ID NO: 425 - protein, 7 aa, synthetic construct
RTSNLAS

SEQ ID NO: 426 - protein, 11 aa, synthetic construct
QQGSSIPRMLT

SEQ ID NO: 427 - protein, 6 aa, synthetic construct
SGYYWI

SEQ ID NO: 428 - protein, 16 aa, synthetic construct
YISYDASNKYKPSLKN

SEQ ID NO: 429 - protein, 9 aa, synthetic construct
EDLRGYFDV

SEQ ID NO: 430 - protein, 15 aa, synthetic construct
RASQSVSTSGFSYMH

SEQ ID NO: 431 - protein, 7 aa, synthetic construct
YASILQS

SEQ ID NO: 432 - protein, 9 aa, synthetic construct
QHSWGIPFT

SEQ ID NO: 433 - protein, 330 aa, synthetic construct
ASTKGPSVFPLAPSSKSTSGGTAALGCLVKDYFPEPVTVSWNSGALTSGVHTFPAVLQSSGLYSLSSVVTVPSSSLGTQTYICNVNHKPSNTKVDKKVEPKSCDKTHTCPPCPAPELLGGPSVFLFPPKPKDTLMISRTPEVTCVVVDVSHEDPEVKFNWYVDGVEVHNAKTKPREEQYNSTYRVVSVLTVLHQDWLNGKEYKCKVSNKALPAPIEKTISKAKGQPREPQVYTLPPSREEMTKNQVSLTCLVKGFYPSDIAVEWESNGQPENNYKTTPPVLDSDGSFFLYSKLTVDKSRWQQGNVFSCSVMHEALHNHYTQKSLSLSPGK

SEQ ID NO: 434 - protein, 107 aa, synthetic construct [sequence omitted]

SEQ ID NO: 435 - protein, 106 aa, synthetic construct
GQPKANPTVTLFPPSSEELQANKATLVCLISDFYPGAVTVAWKADGSPVKAGVETTKPSKQSNNKYAASSYLSLTPEQWKSHRSYSCQVTHEGSTVEKTVAPTECS

SEQ ID NO: 436 - protein, 110 aa, synthetic construct
EIVLTQSPATLSLSPGERATLSCSASSSISSNYLHWYQQKPGQAPRFLIYRTSNLASGIPARFSGSGSGTDFTLTISSLEPEDFAVYYCQQASSIPRMFTFGQGTKLEIK

SEQ ID NO: 437 - protein, 110 aa, synthetic construct
EIVLTQSPDFQSVTPKEKVTITCSASSSISSNYLHWYQQKPDQSPKLLIKRTSNLASGVPSRFSGSGSGTDFTLTINSLEAEDAATYYCQQASSIPRMFTFGQGTKLEIK

SEQ ID NO: 438 - protein, 110 aa, synthetic construct
EIVLTQSPDFQSVTPKEKVTITCSASSSISSNYLHWYQQKPDQSPKFLIYRTSNLASGVPSRFSGSGSGTDFTLTINSLEAEDAATYYCQQASSIPRMFTFGQGTKLEIK

SEQ ID NO: 439 - protein, 119 aa, synthetic construct
EVQLVQSGAEVKKPGASVKVSCKASGYTFTNYWMHWVRQAPGQRLEWMGEIDPSDNYANYNQEFQGRVTITVDKSASTAYMELSSLRSEDTAVYYCARHDGYFGALDYWGQGTTVTVSS

SEQ ID NO: 440 - protein, 119 aa, synthetic construct
EVQLVQSGAEVKKPGASVKVSCKASGYTFTNYWMHWVRQAPGQGLEWMGEIDPSDNYANYNQEFQGRVTITVDKSASTAYMELSSLRSEDTAVYYCARHDGYFGALDYWGQGTTVTVSS

SEQ ID NO: 441 - protein, 119 aa, synthetic construct
EVQLVQSGAEVKKPGASVKVSCKASGYTFTNYWMHWVRQRPGQGLEWMGEIDPSDNYANYNQEFQGRVTITVDKSASTAYMELSSLRSEDTAVYYCARHDGYFGALDYWGQGTTVTVSS

SEQ ID NO: 442 - protein, 119 aa, synthetic construct
EVQLQQSGAEVKKPGASVKVSCKASGYTFTNYWMHWVRQRPGQGLEWMGEIDPSDNYANYNQEFQGRVTITVDKSASTAYMELSSLRSEDTAVYYCARHDGYFGALDYWGQGTTVTVSS

SEQ ID NO: 443 - protein, 95 aa, synthetic construct
EIVLTQSPDFQSVTPKEKVTITCRASQSIGSSLHWYQQKPDQSPKLLIKYASQSFSGVPSRFSGSGSGTDFTLTINSLEAEDAATYYCHQSSSLP

SEQ ID NO: 444 - protein, 95 aa, synthetic construct
EIVLTQSPATLSLSPGERATLSCRASQSVSSYLAWYQQKPGQAPRLLIYDASNRATGIPARFSGSGSGTDFTLTISSLEPEDFAVYYCQQRSNWP

SEQ ID NO: 445 - protein, 10 aa, synthetic construct
FGQGTKLEIK

SEQ ID NO: 446 - protein, 98 aa, synthetic construct
QVQLVQSGAEVKKPGASVKVSCKASGYTFTSYAMHWVRQAPGQRLEWMGWINAGNGNTKYSQKFQGRVTITRDTSASTAYMELSSLRSEDTAVYYCAR

SEQ ID NO: 447 - protein, 11 aa, synthetic construct
WGQGTTVTVSS

SEQ ID NO: 448 - protein, 324 aa, synthetic construct
AKTTPPSVYPLAPGSAAQTNSMVTLGCLVKGYFPEPVTVTWNSGSLSSGVHTFPAVLQSDLYTLSSSVTVPSSTWPSETVTCNVAHPASSTKVDKKIVPRDCGCKPCICTVPEVSSVFIFPPKPKDVLTITLTPKVTCVVVDISKDDPEVQFSWFVDDVEVHTAQTQPREEQFNSTFRSVSELPIMHQDWLNGKEFKCRVNSAAFPAPIEKTISKTKGRPKAPQVYTIPPPKEQMAKDKVSLTCMITDFFPEDITVEWQWNGQPAENYKNTQPIMDTDGSYFVYSKLNVQKSNWEAGNTFTCSVLHEGLHNHHTEKSLSHSPGK

SEQ ID NO: 449 - protein, 107 aa, synthetic construct
RADAAPTVSIFPPSSEQLTSGGASVVCFLNNFYPKDINVKWKIDGSERQNGVLNSWTDQDSKDSTYSMSSTLTLTKDEYERHNSYTCEATHKTSTSPIVKSFNRNEC